European Patent Specification EP 3 463 430 B1, published January 1, 2025. Title: SERUM ALBUMIN-BINDING FIBRONECTIN TYPE III DOMAINS. Applicant: JANSSEN BIOTECH, INC. DIEM, MICHAEL JACOBS, STEVEN O'NEIL, KARYN RUTKOSKI, THOMAS. Application TO BE ASSIGNED. The sequence listing filed with the application follows.

SEQUENCE LISTING (72 sequences)

SEQ ID NO: 1 - protein, 89 aa, Artificial Sequence
  Description of Artificial Sequence: Synthetic polypeptide
LPAPKNLVVSEVTEDSLRLSWTAPDAAFDSFLIQYQESEKVGEAINLTVPGSERSYDLTGLKPGTEYTVSIYGVKGGHRSNPLSAEFTT

SEQ ID NO: 2 - protein, 88 aa, Artificial Sequence
  Description of Artificial Sequence: Synthetic polypeptide
  MOD_RES (75)..(75): Any amino acid
  MOD_RES (76)..(80): Any amino acid or deleted
LPAPKNLVVSEVTEDSLRLSWTAPDAAFDSFLIQYQESEKVGEAINLTVPGSERSYDLTGLKPGTEYTVSIYGVXXXXXXPLSAEFTT

SEQ ID NO: 3 - protein, 89 aa, Artificial Sequence
  Description of Artificial Sequence: Synthetic polypeptide
  MOD_RES (22)..(27): Ala, Arg, Asn, Asp, Glu, Gln, Gly, His, Ile, Leu, Lys, Phe, Pro, Ser, Thr, Trp, Tyr or Val
  MOD_RES (28)..(28): Phe, Ile, Leu, Val or Tyr
  MOD_RES (29)..(29): Asp, Glu or Thr
  MOD_RES (75)..(79): Ala, Arg, Asn, Asp, Glu, Gln, Gly, His, Ile, Leu, Lys, Phe, Pro, Ser, Thr, Trp, Tyr or Val
  MOD_RES (81)..(82): Ala, Arg, Asn, Asp, Glu, Gln, Gly, His, Ile, Leu, Lys, Phe, Pro, Ser, Thr, Trp, Tyr or Val
LPAPKNLVVSEVTEDSLRLSWXXXXXXXXSFLIQYQESEKVGEAINLTVPGSERSYDLTGLKPGTEYTVSIYGVXXXXXSXXLSAEFTT

SEQ ID NO: 4 - protein, 89 aa, Artificial Sequence
  Description of Artificial Sequence: Synthetic polypeptide
LPAPKNLVVSRVTEDSARLSWTAPDAAFDSFLIQYQESEKVGEAIVLTVPGSERSYDLTGLKPGTEYTVSIYGVKGGHRSNPLSAIFTT

SEQ ID NO: 5 - protein, 97 aa, Artificial Sequence
  Description of Artificial Sequence: Synthetic polypeptide
  MOD_RES (22)..(27): Ala, Asp, Glu, Phe, Gly, His, Ile, Lys, Leu, Asn, Pro, Gln, Arg, Ser, Thr, Val, Trp or Tyr
  MOD_RES (28)..(30): Ala, Asp, Glu, Phe, Gly, His, Ile, Lys, Leu, Asn, Pro, Gln, Arg, Ser, Thr, Val, Trp, Tyr or deleted
  MOD_RES (78)..(84): Ala, Asp, Glu, Phe, Gly, His, Ile, Lys, Leu, Asn, Pro, Gln, Arg, Ser, Thr, Val, Trp or Tyr
  MOD_RES (85)..(87): Ala, Asp, Glu, Phe, Gly, His, Ile, Lys, Leu, Asn, Pro, Gln, Arg, Ser, Thr, Val, Trp, Tyr or deleted
LPAPKNLVVSRVTEDSARLSWXXXXXXXXXFDSFLIQYQESEKVGEAIVLTVPGSERSYDLTGLKPGTEYTVSIYGVXXXXXXXXXXSNPLSAIFTT

SEQ ID NO: 6 - protein, 96 aa, Artificial Sequence
  Description of Artificial Sequence: Synthetic polypeptide
  MOD_RES (75)..(81): Ala, Asp, Glu, Phe, Gly, His, Ile, Lys, Leu, Asn, Pro, Gln, Arg, Ser, Thr, Val, Trp or Tyr
  MOD_RES (82)..(86): Ala, Asp, Glu, Phe, Gly, His, Ile, Lys, Leu, Asn, Pro, Gln, Arg, Ser, Thr, Val, Trp, Tyr or deleted
LPAPKNLVVSRVTEDSARLSWTAPDAAFDSFLIQYQESEKVGEAIVLTVPGSERSYDLTGLKPGTEYTVSIYGVXXXXXXXXXXXXSNPLSAIFTT

SEQ ID NO: 7 - protein, 89 aa, Artificial Sequence
  Description of Artificial Sequence: Synthetic polypeptide
  MOD_RES (32)..(32): Ala, Asp, Glu, Phe, Gly, His, Ile, Lys, Leu, Asn, Pro, Gln, Arg, Ser, Thr, Val, Trp, Tyr or Met
  MOD_RES (34)..(34): Ala, Asp, Glu, Phe, Gly, His, Ile, Lys, Leu, Asn, Pro, Gln, Arg, Ser, Thr, Val, Trp, Tyr or Met
  MOD_RES (36)..(36): Ala, Asp, Glu, Phe, Gly, His, Ile, Lys, Leu, Asn, Pro, Gln, Arg, Ser, Thr, Val, Trp, Tyr or Met
  MOD_RES (38)..(40): Ala, Asp, Glu, Phe, Gly, His, Ile, Lys, Leu, Asn, Pro, Gln, Arg, Ser, Thr, Val, Trp, Tyr or Met
  MOD_RES (41)..(41): Any amino acid
  MOD_RES (68)..(68): Any amino acid
  MOD_RES (70)..(70): Any amino acid
  MOD_RES (72)..(72): Ala, Asp, Glu, Phe, Gly, His, Ile, Lys, Leu, Asn, Pro, Gln, Arg, Ser, Thr, Val, Trp, Tyr or Met
  MOD_RES (78)..(79): Ala, Asp, Glu, Phe, Gly, His, Ile, Lys, Leu, Asn, Pro, Gln, Arg, Ser, Thr, Val, Trp, Tyr or Met
  MOD_RES (81)..(81): Ala, Asp, Glu, Phe, Gly, His, Ile, Lys, Leu, Asn, Pro, Gln, Arg, Ser, Thr, Val, Trp, Tyr or Met
LPAPKNLVVSRVTEDSARLSWTAPDAAFDSFXIXYXEXXXXGEAIVLTVPGSERSYDLTGLKPGTEYXVXIXGVKGGXXSXPLSAIFTT

SEQ ID NO: 8 - protein, 89 aa, Artificial Sequence
  Description of Artificial Sequence: Synthetic polypeptide
  MOD_RES (32)..(32): Ala, Asp, Glu, Phe, Gly, His, Ile, Lys, Leu, Asn, Pro, Gln, Arg, Ser, Thr, Val or Trp
  MOD_RES (34)..(34): Ala, Asp, Glu, Phe, Gly, His, Ile, Lys, Leu, Asn, Pro, Gln, Arg, Ser, Thr, Val or Trp
  MOD_RES (36)..(36): Ala, Asp, Glu, Phe, Gly, His, Ile, Lys, Leu, Asn, Pro, Gln, Arg, Ser, Thr, Val or Trp
  MOD_RES (38)..(40): Ala, Asp, Glu, Phe, Gly, His, Ile, Lys, Leu, Asn, Pro, Gln, Arg, Ser, Thr, Val or Trp
  MOD_RES (41)..(41): Any amino acid
  MOD_RES (46)..(46): Any amino acid
  MOD_RES (48)..(48): Any amino acid
  MOD_RES (68)..(68): Ala, Asp, Glu, Phe, Gly, His, Ile, Lys, Leu, Asn, Pro, Gln, Arg, Ser, Thr, Val or Trp
  MOD_RES (70)..(70): Ala, Asp, Glu, Phe, Gly, His, Ile, Lys, Leu, Asn, Pro, Gln, Arg, Ser, Thr, Val or Trp
  MOD_RES (72)..(72): Ala, Asp, Glu, Phe, Gly, His, Ile, Lys, Leu, Asn, Pro, Gln, Arg, Ser, Thr, Val or Trp
  MOD_RES (78)..(78): Ala, Asp, Glu, Phe, Gly, His, Ile, Lys, Leu, Asn, Pro, Gln, Arg, Ser, Thr, Val or Trp
  MOD_RES (79)..(79): Any amino acid
  MOD_RES (81)..(81): Any amino acid
  MOD_RES (84)..(84): Any amino acid
  MOD_RES (86)..(86): Any amino acid
LPAPKNLVVSRVTEDSARLSWTAPDAAFDSFXIXYXEXXXXGEAIXLXVPGSERSYDLTGLKPGTEYXVXIXGVKGGXXSXPLXAXFTT

SEQ ID NO: 9 - DNA, 19 bp, Artificial Sequence
  Description of Artificial Sequence: Synthetic primer
gtgacacggcggttagaac

SEQ ID NO: 10 - DNA, 20 bp, Artificial Sequence
  Description of Artificial Sequence: Synthetic primer
gcctttgggaagcttctaag

SEQ ID NO: 11 - DNA, 30 bp, Artificial Sequence
  Description of Artificial Sequence: Synthetic primer
cggcggttagaacgcggctacaattaatac

SEQ ID NO: 12 - DNA, 22 bp, Artificial Sequence
  Description of Artificial Sequence: Synthetic primer
catgattacgccaagctcagaa

SEQ ID NO: 13 - DNA, 385 bp, Artificial Sequence
  Description of Artificial Sequence: Synthetic polynucleotide
  modified_base (198)..(224): a, c, t, g, unknown or other
gtgacacggcggttagaacgcggctacaattaatacataaccccatccccctgttgacaattaatcatcggctcgtataatgtgtggaattgtgagcggataacaatttcacacaggaaacaggatctaccatgctgccggcgccgaaaaacctggttgtttctgaagttaccgaagactctctgcgtctgtcttggnnnnnnnnnnnnnnnnnnnnnnnnnnnttygactctttcctgatccagtaccaggaatctgaaaaagttggtgaagcgatcaacctgaccgttccgggttctgaacgttcttacgacctgaccggtctgaaaccgggtaccgaatacaccgtttctatctacggtgttcttagaagcttcccaaaggc

SEQ ID NO: 14 - DNA, 382 bp, Artificial Sequence
  Description of Artificial Sequence: Synthetic polynucleotide
  modified_base (198)..(221): a, c, t, g, unknown or other
gtgacacggcggttagaacgcggctacaattaatacataaccccatccccctgttgacaattaatcatcggctcgtataatgtgtggaattgtgagcggataacaatttcacacaggaaacaggatctaccatgctgccggcgccgaaaaacctggttgtttctgaagttaccgaagactctctgcgtctgtcttggnnnnnnnnnnnnnnnnnnnnnnnnttygactctttcctgatccagtaccaggaatctgaaaaagttggtgaagcgatcaacctgaccgttccgggttctgaacgttcttacgacctgaccggtctgaaaccgggtaccgaatacaccgtttctatctacggtgttcttagaagcttcccaaaggc

SEQ ID NO: 15 - DNA, 379 bp, Artificial Sequence
  Description of Artificial Sequence: Synthetic polynucleotide
  modified_base (198)..(218): a, c, t, g, unknown or other
gtgacacggcggttagaacgcggctacaattaatacataaccccatccccctgttgacaattaatcatcggctcgtataatgtgtggaattgtgagcggataacaatttcacacaggaaacaggatctaccatgctgccggcgccgaaaaacctggttgtttctgaagttaccgaagactctctgcgtctgtcttggnnnnnnnnnnnnnnnnnnnnnttygactctttcctgatccagtaccaggaatctgaaaaagttggtgaagcgatcaacctgaccgttccgggttctgaacgttcttacgacctgaccggtctgaaaccgggtaccgaatacaccgtttctatctacggtgttcttagaagcttcccaaaggc

SEQ ID NO: 16 - DNA, 376 bp, Artificial Sequence
  Description of Artificial Sequence: Synthetic polynucleotide
  modified_base (198)..(215): a, c, t, g, unknown or other
gtgacacggcggttagaacgcggctacaattaatacataaccccatccccctgttgacaattaatcatcggctcgtataatgtgtggaattgtgagcggataacaatttcacacaggaaacaggatctaccatgctgccggcgccgaaaaacctggttgtttctgaagttaccgaagactctctgcgtctgtcttggnnnnnnnnnnnnnnnnnnttygactctttcctgatccagtaccaggaatctgaaaaagttggtgaagcgatcaacctgaccgttccgggttctgaacgttcttacgacctgaccggtctgaaaccgggtaccgaatacaccgtttctatctacggtgttcttagaagcttcccaaaggc

SEQ ID NO: 17 - DNA, 131 bp, Artificial Sequence
  Description of Artificial Sequence: Synthetic polynucleotide
cggcggttagaacgcggctacaattaatacataaccccatccccctgttgacaattaatcatcggctcgtataatgtgtggaattgtgagcggataacaatttcacacaggaaacaggatctaccatgctg

SEQ ID NO: 18 - DNA, 30 bp, Artificial Sequence; identical to SEQ ID NO: 11
  Description of Artificial Sequence: Synthetic primer

SEQ ID NO: 19 - DNA, 81 bp, Artificial Sequence
  Description of Artificial Sequence: Synthetic primer
ccaagacagacgggcagagtcttcggtaacgcgagaaacaaccaggtttttcggcgccggcagcatggtagatcctgtttc

SEQ ID NO: 20 - DNA, 26 bp, Artificial Sequence
  Description of Artificial Sequence: Synthetic oligonucleotide
ccgaagactctgcccgtctgtcttgg

SEQ ID NO: 21 - DNA, 45 bp, Artificial Sequence
  Description of Artificial Sequence: Synthetic oligonucleotide
cagtggtctcacggattcctggtactggatcaggaaagagtcgaa

SEQ ID NO: 22 - DNA, 54 bp, Artificial Sequence
  Description of Artificial Sequence: Synthetic oligonucleotide
catgcggtctcttccgaaaaagttggtgaagcgatcgtcctgaccgttccgggt

SEQ ID NO: 23 - DNA, 29 bp, Artificial Sequence
  Description of Artificial Sequence: Synthetic oligonucleotide
ggtggtgaagatcgcagacagcgggttag

SEQ ID NO: 24 - DNA, 21 bp, Artificial Sequence
  Description of Artificial Sequence: Synthetic oligonucleotide
cggcggttagaacgcggctac

SEQ ID NO: 25 - DNA, 61 bp, Artificial Sequence
  Description of Artificial Sequence: Synthetic oligonucleotide
aagatcagttgcggccgctagactagaaccgctgccaccgccggtggtgaagatcgcagac

SEQ ID NO: 26 - DNA, 485 bp, Artificial Sequence
  Description of Artificial Sequence: Synthetic polynucleotide
  modified_base (357)..(392): a, c, t, g, unknown or other
gtgacacggcggttagaacgcggctacaattaatacataaccccatccccctgttgacaattaatcatcggctcgtataatgtgtggaattgtgagcggataacaatttcacacaggaaacaggatctaccatgctgccggcgccgaaaaacctggttgtttctcgcgttaccgaagactctgcgcgtctgtcttggaccgcgccggacgcggcgttcgactctttcctgatccagtaccaggaatctgaaaaagttggtgaagcgatcgtgctgaccgttccgggttctgaacgttcttacgacctgaccggtctgaaaccgggtaccgaatacaccgtttctatctacggtgttnnnnnnnnnnnnnnnnnnnnnnnnnnnnnnnnnnnntctaacccgctgtctgcgatcttcaccaccggcggtcaccatcaccatcaccatggcagcggttctagtctagcggccgcaactgatcttggc

SEQ ID NO: 27 - DNA, 482 bp, Artificial Sequence
  Description of Artificial Sequence: Synthetic polynucleotide
  modified_base (357)..(389): a, c, t, g, unknown or other
gtgacacggcggttagaacgcggctacaattaatacataaccccatccccctgttgacaattaatcatcggctcgtataatgtgtggaattgtgagcggataacaatttcacacaggaaacaggatctaccatgctgccggcgccgaaaaacctggttgtttctcgcgttaccgaagactctgcgcgtctgtcttggaccgcgccggacgcggcgttcgactctttcctgatccagtaccaggaatctgaaaaagttggtgaagcgatcgtgctgaccgttccgggttctgaacgttcttacgacctgaccggtctgaaaccgggtaccgaatacaccgtttctatctacggtgttnnnnnnnnnnnnnnnnnnnnnnnnnnnnnnnnntctaacccgctgtctgcgatcttcaccaccggcggtcaccatcaccatcaccatggcagcggttctagtctagcggccgcaactgatcttggc

SEQ ID NO: 28 - DNA, 479 bp, Artificial Sequence
  Description of Artificial Sequence: Synthetic polynucleotide
  modified_base (357)..(386): a, c, t, g, unknown or other
gtgacacggcggttagaacgcggctacaattaatacataaccccatccccctgttgacaattaatcatcggctcgtataatgtgtggaattgtgagcggataacaatttcacacaggaaacaggatctaccatgctgccggcgccgaaaaacctggttgtttctcgcgttaccgaagactctgcgcgtctgtcttggaccgcgccggacgcggcgttcgactctttcctgatccagtaccaggaatctgaaaaagttggtgaagcgatcgtgctgaccgttccgggttctgaacgttcttacgacctgaccggtctgaaaccgggtaccgaatacaccgtttctatctacggtgttnnnnnnnnnnnnnnnnnnnnnnnnnnnnnntctaacccgctgtctgcgatcttcaccaccggcggtcaccatcaccatcaccatggcagcggttctagtctagcggccgcaactgatcttggc

SEQ ID NO: 29 - DNA, 476 bp, Artificial Sequence
  Description of Artificial Sequence: Synthetic polynucleotide
  modified_base (357)..(383): a, c, t, g, unknown or other
gtgacacggcggttagaacgcggctacaattaatacataaccccatccccctgttgacaattaatcatcggctcgtataatgtgtggaattgtgagcggataacaatttcacacaggaaacaggatctaccatgctgccggcgccgaaaaacctggttgtttctcgcgttaccgaagactctgcgcgtctgtcttggaccgcgccggacgcggcgttcgactctttcctgatccagtaccaggaatctgaaaaagttggtgaagcgatcgtgctgaccgttccgggttctgaacgttcttacgacctgaccggtctgaaaccgggtaccgaatacaccgtttctatctacggtgttnnnnnnnnnnnnnnnnnnnnnnnnnnntctaacccgctgtctgcgatcttcaccaccggcggtcaccatcaccatcaccatggcagcggttctagtctagcggccgcaactgatcttggc

SEQ ID NO: 30 - DNA, 473 bp, Artificial Sequence
  Description of Artificial Sequence: Synthetic polynucleotide
  modified_base (357)..(380): a, c, t, g, unknown or other
gtgacacggcggttagaacgcggctacaattaatacataaccccatccccctgttgacaattaatcatcggctcgtataatgtgtggaattgtgagcggataacaatttcacacaggaaacaggatctaccatgctgccggcgccgaaaaacctggttgtttctcgcgttaccgaagactctgcgcgtctgtcttggaccgcgccggacgcggcgttcgactctttcctgatccagtaccaggaatctgaaaaagttggtgaagcgatcgtgctgaccgttccgggttctgaacgttcttacgacctgaccggtctgaaaccgggtaccgaatacaccgtttctatctacggtgttnnnnnnnnnnnnnnnnnnnnnnnntctaacccgctgtctgcgatcttcaccaccggcggtcaccatcaccatcaccatggcagcggttctagtctagcggccgcaactgatcttggc

SEQ ID NO: 31 - DNA, 470 bp, Artificial Sequence
  Description of Artificial Sequence: Synthetic polynucleotide
  modified_base (357)..(377): a, c, t, g, unknown or other
gtgacacggcggttagaacgcggctacaattaatacataaccccatccccctgttgacaattaatcatcggctcgtataatgtgtggaattgtgagcggataacaatttcacacaggaaacaggatctaccatgctgccggcgccgaaaaacctggttgtttctcgcgttaccgaagactctgcgcgtctgtcttggaccgcgccggacgcggcgttcgactctttcctgatccagtaccaggaatctgaaaaagttggtgaagcgatcgtgctgaccgttccgggttctgaacgttcttacgacctgaccggtctgaaaccgggtaccgaatacaccgtttctatctacggtgttnnnnnnnnnnnnnnnnnnnnntctaacccgctgtctgcgatcttcaccaccggcggtcaccatcaccatcaccatggcagcggttctagtctagcggccgcaactgatcttggc

SEQ ID NO: 32 - protein, 7 aa, Artificial Sequence
  Description of Artificial Sequence: Synthetic peptide
KGGHRSN

SEQ ID NO: 33 - DNA, 37 bp, Artificial Sequence
  Description of Artificial Sequence: Synthetic oligonucleotide
aagaaggagaaccggtatgctgccggcgccgaaaaac

SEQ ID NO: 34 - DNA, 65 bp, Artificial Sequence
  Description of Artificial Sequence: Synthetic oligonucleotide
gagccgccgccaccggtttaatggtgatggtgatggtgaccaccggtggtgaagatcgcagacag

SEQ ID NO: 35 - protein, 8 aa, Homo sapiens
SFLIQYQE

SEQ ID NO: 36 - protein, 8 aa, Artificial Sequence
  Description of Artificial Sequence: Synthetic peptide
SFQIEYWE

SEQ ID NO: 37 - protein, 8 aa, Artificial Sequence
  Description of Artificial Sequence: Synthetic peptide
SFKILYEE

SEQ ID NO: 38 - protein, 8 aa, Artificial Sequence
  Description of Artificial Sequence: Synthetic peptide
SFHIEYWE

SEQ ID NO: 39 - protein, 6 aa, Homo sapiens
SEKVGE

SEQ ID NO: 40 - protein, 6 aa, Artificial Sequence
  Description of Artificial Sequence: Synthetic peptide
DDVGGE

SEQ ID NO: 41 - protein, 6 aa, Artificial Sequence
  Description of Artificial Sequence: Synthetic peptide
YLVFGE

SEQ ID NO: 42 - protein, 6 aa, Artificial Sequence
  Description of Artificial Sequence: Synthetic peptide
QSIVGE

SEQ ID NO: 43 - protein, 10 aa, Homo sapiens
EYTVSIYGVK

SEQ ID NO: 44 - protein, 10 aa, Artificial Sequence
  Description of Artificial Sequence: Synthetic peptide
EYDVYILGVK

SEQ ID NO: 45 - protein, 10 aa, Artificial Sequence
  Description of Artificial Sequence: Synthetic peptide
EYWVAIWGVK

SEQ ID NO: 46 - protein, 10 aa, Artificial Sequence
  Description of Artificial Sequence: Synthetic peptide
EYRVWIYGVK

SEQ ID NO: 47 - protein, 7 aa, Homo sapiens
GGHRSNP

SEQ ID NO: 48 - protein, 7 aa, Artificial Sequence
  Description of Artificial Sequence: Synthetic peptide
GGWESGP

SEQ ID NO: 49 - protein, 7 aa, Artificial Sequence
  Description of Artificial Sequence: Synthetic peptide
GGQVSGT

SEQ ID NO: 50 - protein, 7 aa, Artificial Sequence
  Description of Artificial Sequence: Synthetic peptide
GGNDSWP

SEQ ID NO: 51 - protein, 89 aa, Artificial Sequence
  Description of Artificial Sequence: Synthetic polypeptide
LPAPKNLVVSRVTEDSARLSWTAPDAAFDSFQIEYWEDDVGGEAIVLTVPGSERSYDLTGLKPGTEYDVYILGVKGGWESGPLSAIFTT

SEQ ID NO: 52 - protein, 89 aa, Artificial Sequence
  Description of Artificial Sequence: Synthetic polypeptide
LPAPKNLVVSRVTEDSARLSWTAPDAAFDSFKILYEEYLVFGEAIVLTVPGSERSYDLTGLKPGTEYWVAIWGVKGGQVSGTLSAIFTT

SEQ ID NO: 53 - protein, 89 aa, Artificial Sequence
  Description of Artificial Sequence: Synthetic polypeptide
LPAPKNLVVSRVTEDSARLSWTAPDAAFDSFHIEYWEQSIVGEAIVLTVPGSERSYDLTGLKPGTEYRVWIYGVKGGNDSWPLSAIFTT

SEQ ID NO: 54 - protein, 4 aa, Artificial Sequence
  Description of Artificial Sequence: Synthetic peptide
GSGS

SEQ ID NO: 55 - protein, 8 aa, Artificial Sequence
  Description of Artificial Sequence: Synthetic peptide
GGGSGGGS

SEQ ID NO: 56 - protein, 25 aa, Artificial Sequence
  Description of Artificial Sequence: Synthetic peptide
GGGGSGGGGSGGGGSGGGGSGGGGS

SEQ ID NO: 57 - protein, 4 aa, Artificial Sequence
  Description of Artificial Sequence: Synthetic peptide
APAP

SEQ ID NO: 58 - protein, 10 aa, Artificial Sequence
  Description of Artificial Sequence: Synthetic peptide
APAPAPAPAP

SEQ ID NO: 59 - protein, 20 aa, Artificial Sequence
  Description of Artificial Sequence: Synthetic peptide
APAPAPAPAPAPAPAPAPAP

SEQ ID NO: 60 - protein, 40 aa, Artificial Sequence
  Description of Artificial Sequence: Synthetic polypeptide
APAPAPAPAPAPAPAPAPAPAPAPAPAPAPAPAPAPAPAP

SEQ ID NO: 61 - protein, 29 aa, Artificial Sequence
  Description of Artificial Sequence: Synthetic peptide
AEAAAKEAAAKEAAAKEAAAKEAAAKAAA

SEQ ID NO: 62 - protein, 608 aa, Homo sapiens
KWVTFISLLFLFSSAYSRGVFRRDAHKSEVAHRFKDLGEENFKALVLIAFAQYLQQCPFEDHVKLVNEVTEFAKTCVADESAENCDKSLHTLFGDKLCTVATLRETYGEMADCCAKQEPERNECFLQHKDDNPNLPRLVRPEVDVMCTAFHDNEETFLKKYLYEIARRHPYFYAPELLFFAKRYKAAFTECCQAADKAACLLPKLDELRDEGKASSAKQRLKCASLQKFGERAFKAWAVARLSQRFPKAEFAEVSKLVTDLTKVHTECCHGDLLECADDRADLAKYICENQDSISSKLKECCEKPLLEKSHCIAEVENDEMPADLPSLAADFVESKDVCKNYAEAKDVFLGMFLYEYARRHPDYSVVLLLRLAKTYETTLEKCCAAADPHECYAKVFDEFKPLVEEPQNLIKQNCELFEQLGEYKFQNALLVRYTKKVPQVSTPTLVEVSRNLGKVGSKCCKHPEAKRMPCAEDYLSVVLNQLCVLHEKTPVSDRVTKCCTESLVNRRPCFSALEVDETYVPKEFNAETFTFHADICTLSEKERQIKKQTALVELVKHKPKATKEQLKAVMDDFAAFVEKCCKADDKETCFAEEGKKLVAASQAALGL

SEQ ID NO: 63 - protein, 607 aa, Macaca mulatta
KWVTFISLLFLFSSAYSRGVFRRDTHKSEVAHRFKDLGEEHFKGLVLVAFSQYLQQCPFEEHVKLVNEVTEFAKTCVADESAENCDKSLHTLFGDKLCTVATLRETYGEMADCCAKQEPERNECFLQHKDDNPNLPPLVRPEVDVMCTAFHDNEATFLKKYLYEVARRHPYFYAPELLFFAARYKAAFAECCQAADKAACLLPKLDELRDEGKASSAKQRLKCASLQKFGDRAFKAWAVARLSQKFPKAEFAEVSKLVTDLTKVHTECCHGDLLECADDRADLAKYMCENQDSISSKLKECCDKPLLEKSHCLAEVENDEMPADLPSLAADYVESKDVCKNYAEAKDVFLGMFLYEYARRHPDYSVMLLLRLAKAYEATLEKCCAAADPHECYAKVFDEFQPLVEEPQNLVKQNCELFEQLGEYKFQNALLVRYTKKVPQVSTPTLVEVSRNLGKVGAKCCKLPEAKRMPCAEDYLSVVLNRLCVLHEKTPVSEKVTKCCTESLVNRRPCFSALELDEAYVPKAFNAETFTFHADMCTLSEKEKQVKKQTALVELVKHKPKATKEQLKGVMDNFAAFVEKCCKADDKEACFAEEGPKFVAASQAALA

SEQ ID NO: 64 - DNA, 267 bp, Artificial Sequence
  Description of Artificial Sequence: Synthetic polynucleotide
ttgccggccccgaagaacctggtcgtgagccgtgttaccgaggacagcgcgcgtctgagctggaccgcaccggacgcggcgtttgattcgtttcagattgagtattgggaagatgacgtgggtggtgaggctatcgtgctgaccgtcccgggtagcgagcgcagctacgatctgacgggtctgaaaccgggtaccgagtacgacgtgtacattttgggtgttaaaggtggctgggagagcggtccgctgtcagcaatctttacgacg

SEQ ID NO: 65 - DNA, 267 bp, Artificial Sequence
  Description of Artificial Sequence: Synthetic polynucleotide
ctgccggccccgaagaacctggtcgtgagccgtgttaccgaggacagcgcgcgtctgagctggaccgcaccggacgcggcgtttgattcgtttaagattctgtatgaagaatacctggtgttcggtgaggctatcgtgctgaccgtcccgggtagcgagcgcagctacgatctgacgggtctgaaaccgggtaccgagtactgggtggcgatttggggtgttaaaggtggccaggtgagcggcaccctgagcgcaatctttacgacg

SEQ ID NO: 66 - DNA, 270 bp, Artificial Sequence
  Description of Artificial Sequence: Synthetic polynucleotide
atgttgccggccccgaagaacctggtcgtgagccgtgttaccgaggacagcgcgcgtctgagctggaccgcaccggacgcggcgtttgattcgtttcacattgagtattgggaacagagcatcgtgggtgaggctatcgtgctgaccgtcccgggtagcgagcgcagctacgatctgacgggtctgaaaccgggtaccgagtaccgcgtgtggatttacggtgttaaaggtggcaatgacagctggccgctgtcagcaatctttacgacg

SEQ ID NO: 67 - protein, 89 aa, Artificial Sequence
  Description of Artificial Sequence: Synthetic polypeptide
LPAPKNLVVSEVTEDSARLSWTAPDAAFDSFLIQYQESEKVGEAIVLTVPGSERSYDLTGLKPGTEYTVSIYGVKGGHRSNPLSAIFTT

SEQ ID NO: 68 - protein, 88 aa, Homo sapiens
DAPSQIEVKDVTDTTALITWFKPLAEIDGIELTYGIKDVPGDRTTIDLTEDENQYSIGNLKPDTEYEVSLISRRGDMSSNPAKETFTT

SEQ ID NO: 69 - protein, 89 aa, Artificial Sequence
  Description of Artificial Sequence: Synthetic polypeptide
LDAPTDLQVTNVTDTSITVSWTPPSATITGYRITYTPSNGPGEPKELTVPPSSTSVTITGLTPGVEYVVSLYALKDNQESPPLVGTQTT

SEQ ID NO: 70 - protein, 94 aa, Homo sapiens
VSDVPRDLEVVAATPTSLLISWDAPAVTVRYYRITYGETGGNSPVQEFTVPGSKSTATISGLKPGVDYTITVYAVTGRGDSPASSKPISINYRT

SEQ ID NO: 71 - protein, 20 aa, Artificial Sequence
  Description of Artificial Sequence: Synthetic peptide
GGGGSGGGGSGGGGSGGGGS

SEQ ID NO: 72 - protein, 6 aa, Artificial Sequence
  Description of Artificial Sequence: Synthetic 6xHis tag
HHHHHH